European Patent Application EP 4 755 914 A1, published June 10, 2026. Title: 一种抗ROR1蛋白的抗体及其缀合物. Applicant: 石药集团巨石生物制药有限公司. The sequence listing filed with the application follows.

SEQUENCE LISTING (31 sequences)

SEQ ID NO: 1 - protein, 7 aa, synthetic construct
TSGMGVA

SEQ ID NO: 2 - protein, 16 aa, synthetic construct
HIWWDDDKRYNPSLKS

SEQ ID NO: 3 - protein, 16 aa, synthetic construct
PQFITTVVAFYWYFDV

SEQ ID NO: 4 - protein, 11 aa, synthetic construct
RASENIYSNLA

SEQ ID NO: 5 - protein, 7 aa, synthetic construct
AATNLAD

SEQ ID NO: 6 - protein, 9 aa, synthetic construct
QHFWGTPWT

SEQ ID NO: 7 - protein, 126 aa, synthetic construct
QVTLKESGPTLVKPTQTLTLTCSFSGFSLSTSGMGVAWIRQPPGKALEWLAHIWWDDDKRYNPSLKSRLTITKDTSKNQVVLTMTNMDPVDTATYYCARPQFITTVVAFYWYFDVWGQGTTVTVSS

SEQ ID NO: 8 - protein, 107 aa, synthetic construct
DILLTQSPSSLSVSVGDRVTITCRASENIYSNLAWYQQKPGKAPKLLVYAATNLADGVPSRFSGSGSGTQYTLTISSLQPEDFATYYCQHFWGTPWTFGGGTKLEIK

SEQ ID NO: 9 - protein, 16 aa, synthetic construct
HIWWDDDKRYNPALKS

SEQ ID NO: 10 - protein, 126 aa, synthetic construct
EVTLKESGPTLVKPTQTLTLTCSFSGFSLSTSGMGVAWIRQPPGKALEWLAHIWWDDDKRYNPALKSRLTITKDTSKNQVVLTITNVDPVDTATYYCARPQFITTVVAFYWYFDVWGQGTTVTVSS

SEQ ID NO: 11 - protein, 16 aa, synthetic construct
HIWWDDDKRYGPSLKS

SEQ ID NO: 12 - protein, 126 aa, synthetic construct
QVTLKESGPTLVKPTQTLTLTCTFSGFSLSTSGMGVAWIRQPPGKALEWLAHIWWDDDKRYGPSLKSRLTITKDTSKNQVVLTMTNMDPVDTATYYCARPQFITTVVAFYWYFDVWGQGTTVTVSS

SEQ ID NO: 13 - protein, 330 aa, synthetic construct
ASTKGPSVFPLAPSSKSTSGGTAALGCLVKDYFPEPVTVSWNSGALTSGVHTFPAVLQSSGLYSLSSVVTVPSSSLGTQTYICNVNHKPSNTKVDKKVEPKSCDKTHTCPPCPAPEAAGGPSVFLFPPKPKDTLMISRTPEVTCVVVDVSHEDPEVKFNWYVDGVEVHNAKTKPREEQYNSTYRVVSVLTVLHQDWLNGKEYKCKVSNKALAASIEKTISKAKGQPREPQVYTLPPSRDELTKNQVSLTCLVKGFYPSDIAVEWESNGQPENNYKTTPPVLDSDGSFFLYSKLTVDKSRWQQGNVFSCSVMHEALHNHYTQKSLSLSPGK

SEQ ID NO: 14 - protein, 114 aa, synthetic construct
RTVAAPSVFIFPPSDEQLKSGTASVVCLLNNFYPREAKVQWKVDNALQSGNSQESVTEQDSKDSTYSLSSTLTLSKADYEKHKVYACEVTHQGLSSPVTKSFNRGECGGLQSGA

SEQ ID NO: 15 - protein, 331 aa, synthetic construct
DSDERVTPPAEPLDRMPDPYRPSYGRAETIVNNYIRKWQQVYSHRDGRKQQMTEEQREWLSYGCVGVTWVNSGQYPTNRLAFAFFDEDKYKNELKNGRPRSGETRAEFEGRVAKDSFDEAKGFQRARDVASVMNKALENAHDEGAYLDNLKKELANGNDALRNEDARSPFYSALRNTPSFKDRNGGNHDPSKMKAVIYSKHFWSGQDRSGSSDKRKYGDPEAFRPDRGTGLVDMSRDRNIPRSPTSPGESFVNFDYGWFGAQTEADADKTVWTHGNHYHAPNGSLGAMHVYESKFRNWSDGYSDFDRGAYVVTFVPKSWNTAPDKVTQGWP

SEQ ID NO: 16 - protein, 331 aa, synthetic construct
DSDDRVTPPAEPLDRMPDPYRPSYGRAETVVNNYIRKWQQVYSHRDGRKQQMTEEQREWLSYGCVGVTWVNSGQYPTNRLAFASFDEDRFKNELKNGRPRSGETRAEFEGRVAKESFDEEKGFQRAREVASVMNRALENAHDESAYLDNLKKELANGNDALRNEDARSPFYSALRNTPSFKERNGGNHDPSRMKAVIYSKHFWSGQDRSSSADKRKYGDPDAFRPAPGTGLVDMSRDRNIPRSPTSPGEGFVNFDYGWFGAQTEADADKTVWTHGNHYHAPNGSLGAMHVYESKFRNWSEGYSDFDRGAYVITFIPKSWNTAPDKVKQGWP

SEQ ID NO: 17 - protein, 126 aa, synthetic construct
EVTLKESGPGILQPSQTLSLTCSFSGFSLSTSGMGVAWIRQPSGKGLEWLAHIWWDDDKRYNPALKSRLTISKDTSSNQVFLKIASVDTADTATYYCARPQFITTVVAFYWYFDVWGAGTTVTVSS

SEQ ID NO: 18 - protein, 107 aa, synthetic construct
DILLTQSPASLSVSMGETVTITCRASENIYSNLAWYQQKQGKSPQLLVYAATNLADGVPSRFSGSGSGTQYSLKINSLQSEDFGSYYCQHFWGTPWTFGGGTKLEIK

SEQ ID NO: 19 - protein, 107 aa, synthetic construct [sequence omitted]

SEQ ID NO: 20 - protein, 10 aa, synthetic construct
GFSLSTSGMG

SEQ ID NO: 21 - protein, 7 aa, synthetic construct
IWWDDDK

SEQ ID NO: 22 - protein, 18 aa, unidentified
ARPQFITTVVAFYWYFDV

SEQ ID NO: 23 - protein, 6 aa, synthetic construct
ENIYSN

SEQ ID NO: 24 - protein, 9 aa, synthetic construct
GFSLSTSGM

SEQ ID NO: 25 - protein, 5 aa, synthetic construct
WWDDD

SEQ ID NO: 26 - protein, 8 aa, synthetic construct
STSGMGVA

SEQ ID NO: 27 - protein, 12 aa, synthetic construct
WLAHIWWDDDKR

SEQ ID NO: 28 - protein, 17 aa, synthetic construct
ARPQFITTVVAFYWYFD

SEQ ID NO: 29 - protein, 7 aa, synthetic construct
YSNLAWY

SEQ ID NO: 30 - protein, 10 aa, synthetic construct
LLVYAATNLA

SEQ ID NO: 31 - protein, 8 aa, synthetic construct
QHFWGTPW